European Patent Application EP 4 374 870 A1, published May 29, 2024. Title: Codon-optimized oligonucleotide for induction of elastin de-novo synthesis in mammals. Applicant: Eberhard Karls Universität Tübingen Medizinische Fakultät. Application EP. The sequence listing filed with the application follows.

SEQUENCE LISTING (19 sequences)

SEQ ID NO: 1 - protein, 724 aa, synthetic construct
MAGLTAAAPRPGVLLLLLSILHPSRPGGVPGAIPGGVPGGVFYPGAGLGALGGGALGPGGKPLKPVPGGLAGAGLGAGLGAFPAVTFPGALVPGGVADAAAAYKAAKAGAGLGGVPGVGGLGVSAGAVVPQPGAGVKPGKVPGVGLPGVYPGGVLPGARFPGVGVLPGVPTGAGVKPKAPGVGGAFAGIPGVGPFGGPQPGVPLGYPIKAPKLPGGYGLPYTTGKLPYGYGPGGVAGAAGKAGYPTGTGVGPQAAAAAAAKAAAKFGAGAAGVLPGVGGAGVPGVPGAIPGIGGIAGVGTPAAAAAAAAAAKAAKYGAAAGLVPGGPGFGPGVVGVPGAGVPGVGVPGAGIPVVPGAGIPGAAVPGVVSPEAAAKAAAKAAKYGARPGVGVGGIPTYGVGAGGFPGFGVGVGGIPGVAGVPGVGGVPGVGGVPGVGISPEAQAAAAAKAAKYGVGTPAAAAAKAAAKAAQFGLVPGVGVAPGVGVAPGVGVAPGVGLAPGVGVAPGVGVAPGVGVAPGIGPGGVAAAAKSAAKVAAKAQLRAAAGLGAGIPGLGVGVGVPGLGVGAGVPGLGVGAGVPGFGAVPGALAAAKAAKYGAAVPGVLGGLGALGGVGIPGGVVGAGPAAAAAAAKAAAKAAQFGLVGAAGLGGLGVGGLGVPGVGGLGGIPPAAAAKAAKYGAAGLGGVLGGAGQFPLGGVAARPGFGLSPIFPGGACLGKACGRKRK

SEQ ID NO: 2 - RNA, 2175 nt, synthetic construct
  source 1..2175: mol_type = other RNA
atggccggcctcacagccgccgcccccaggcccggggtgctgctgctgctgctgagcatcctgcaccccagccgccctggcggcgtgcctggcgccatccctggcggggtgcccggcggcgtgttctacccaggagccggcctgggcgccctgggaggcggcgctctgggccccggcgggaagcccctgaagcccgtgcccggcggcctggccggcgccggcctgggggccggcctgggagccttcccagccgtgacattccccggcgccctggtgcccggaggagtggccgacgccgccgccgcctacaaggctgccaaggccggcgctgggctgggcggagtgccaggcgtgggcgggctgggcgtgagtgccggtgccgtggtgccccagcctggagccggcgtgaagcctggcaaagtgcccggagtgggcctgcctggcgtgtatccaggcggcgtcctgccaggcgccaggtttcctggcgtcggcgtgctgcctggcgtgcccactggcgctggcgtgaaacccaaagccccaggcgttggcggggcctttgccggcatccctggagtgggccccttcggcgggccacagcccggagtgccactgggctatcctatcaaagcccccaagctgcctggcggatacgggctcccttacaccaccggcaagctgccctatggctacggccccggcggagtggctggcgccgcagggaaggccggctaccccacaggcaccggcgtggggcctcaggccgctgctgcagccgccgccaaggcagccgccaagttcggggccggggctgccggtgtgctgcccggcgtgggcggagcaggcgtgcccggggtgccaggcgccatcccaggaatcgggggcatcgccggggtgggaacccccgctgccgccgccgctgctgctgccgccgctaaggccgccaaatatggcgccgccgccggactggtgcctgggggcccaggcttcgggcccggcgtggtgggcgtgcctggcgccggcgtgccaggggtgggagtgccaggcgctggcatccctgtggtgcccggagctggcatcccaggagcagccgtgcctggagtggtgtccccagaagccgctgctaaagccgccgccaaggccgccaaatacggtgcccggcccggcgtgggcgtgggcggcattcccacctacggcgtgggcgccgggggcttcccaggctttggggtgggggttggaggcatccctggggtggccggcgtgcctggcgtgggcggcgtccctggggtgggcggcgtgcccggcgtggggatcagccccgaggcccaggccgctgctgccgcaaaagccgccaaatacggagtgggcacccccgccgccgccgccgccaaagccgccgccaaagcagcccagttcggcctggtgcctggagtcggagtggcccctggcgtcggagtggccccaggagtcggagtggcccccggcgtcggcctggctcctggggtgggggtggctccaggcgtgggagtggccccaggcgtgggcgtggcccccggcatcggccccggaggcgtggccgccgccgccaagtccgcagcaaaggtggccgccaaagctcagctgcgcgccgccgccggcctcggcgccggcatccccgggctcggcgtgggcgtgggggtgcctggactgggcgtgggcgccggagtgccaggcctgggggtgggcgccggggtgcccgggtttggggcagtgccaggcgccctggccgccgcaaaagccgcaaagtacggggccgccgtgccaggcgtgctgggtggcctgggcgccctgggcggggtgggcattcccggcggagtggtgggcgccggacctgccgctgccgccgctgctgccaaggccgccgccaaggccgcacagtttggcctggtgggggccgccggcctgggcgggctgggcgtgggcggcctgggcgtgcccggcgtgggcggactgggcggcatcccccctgccgctgccgccaaagctgccaagtacggcgcagccggcctcggcggcgtgctgggcggggccggccagtttccactggggggcgtggccgcccgccccggatttggcctgtctcccatcttccctggcggcgcctgcctgggaaaagcctgtggcaggaagagaaagtga

SEQ ID NO: 3 - RNA, 2175 nt, synthetic construct
  source 1..2175: mol_type = other RNA
atggccggacttaccgctgctgctccaagaccaggagtccttctcctgttattatctattttacacccttcaagacccggaggagttcctggagctattcctggaggggttccaggaggagttttttacccaggggcaggcttaggagccttaggtggtggcgcattagggcctggaggaaaacctctcaaaccagttcctggtggccttgcaggcgctggattaggcgctggactaggggcatttccagcagtgacctttcctggcgcactggtgccagggggagtggcggatgccgccgctgcttataaggctgcaaaagctggtgctggtctgggaggtgttccaggagtgggaggcttgggtgtgtctgccggcgctgtggtaccccagccaggcgcgggagtgaagccaggcaaagtgcccggggtcggcctgcccggcgtgtatcctggcggcgtgctgcctggcgccagatttccaggagtgggcgtgttgcccggcgtccccaccggcgctggtgtcaagcctaaagcacccggtgtggggggggcctttgccgggatccccggggtggggcccttcggcggcccacaaccaggcgtgcccctgggctatcctatcaaagcccccaagctgccaggagggtatgggctgccttacaccacaggcaaactgccctatggctacggcccaggcggcgtcgccggcgccgctgggaaggcgggataccccaccgggacaggcgtcgggccacaggccgctgctgccgcagccgccaaggccgccgccaaattcggcgccggcgccgccggggtgctccccggcgtggggggcgcgggagtgcccggagtgccaggtgccatacccggaattggcggcattgccggggttgggactccagctgccgctgctgcagccgccgctgccgcaaaggccgccaaatatggcgctgccgccgggctcgtccctggcggccctgggtttgggcccggcgtcgtcggcgtcccgggggccggggtgcctggcgtgggggtgccaggagccgggattcctgtggtgcccggggctgggatcccgggcgccgccgttccaggggtcgtaagtcctgaagccgccgctaaagcggccgccaaggccgctaagtatggcgcccgcccaggcgtgggggtgggtgggattcccacctacggcgtcggggcaggggggttccccggctttggtgtcggtgtcggaggaatccccggcgtggccggcgtccccggcgtgggcggggttcccggggtggggggcgtgcctggcgtgggaatctcccccgaggcccaagccgccgccgcggccaaggccgccaagtatggagtcggtacaccagccgccgcagctgcgaaagccgccgccaaagccgcccagttcggccttgtgccgggcgtgggcgtggccccgggggtgggtgtcgcccctggcgtgggtgttgctccaggcgtgggcctggcccccggggtgggcgtggcccctggcgtgggagtggcccccggcgtgggggtggctccaggcattggacccgggggggtggccgccgctgccaagtccgccgccaaggtggcagccaaggctcagctcagggccgccgccggcctcggggccggcatcccgggcctgggcgtgggggtgggcgtgccgggcctgggcgtgggtgccggcgtgcccggcctgggagtgggcgctggggtgcctgggttcggggccgtgcccggcgccctggctgcagccaaggccgccaaatatggagccgccgtccccggggtgctaggcggactgggagccctaggcggagtgggcatccccggcggcgtggtgggtgccggtcccgccgctgccgctgccgctgctaaggccgccgccaaggctgcccagtttggactggtcggcgccgctgggctgggaggcctcggggtgggaggactgggcgtgccaggggtgggggggctgggcgggatccctccagcagctgcggccaaagccgccaaatacggcgccgccggcctgggaggcgtgctgggcggggccggccagtttcccctggggggagtggccgcccgccccggttttggcctgtctcccatcttccccgggggcgcctgcctgggaaaggcctgtggcaggaagagaaagtga

SEQ ID NO: 4 - RNA, 2175 nt, synthetic construct
  source 1..2175: mol_type = other RNA
atggccggcctcaccgccgccgccccccggccgggcgtgctgctgctgctgctgtccatcctgcaccccagccggcccgggggggtgcccggcgccatcccaggaggcgtgccagggggggtcttctacccaggagcaggtctgggcgccctgggtggcggggctctgggccccggcgggaagcccctcaagcccgtcccaggcggcctggccggcgccgggctgggagcaggcctgggcgcgttccctgccgtgaccttccccggggccctggtgcctggcggcgtcgcagacgccgccgccgcctacaaggccgccaaggccggcgctgggctgggcggggtgcccggtgtcgggggattgggagtgtctgccggcgctgtggtgccccagccaggcgccggagtgaagccaggcaaagtgcccggggtcggcctgcccggcgtgtaccctggcggcgtgctgcctggcgccagatttccaggagtgggcgtgttgcctggcgtccccacaggcgccggcgttaagcctaaagcacccggtgtggggggggcctttgccgggatcccaggggtggggcccttcggcggcccacaaccaggcgtgcccctgggctaccctatcaaggcccccaagctgccaggagggtacgggctgccttacaccacaggcaaactgccctatggctacggccccggcggcgtcgccggcgccgctgggaaggcgggataccccaccgggacaggcgtcggccctcaagctgctgccgctgcagctgcaaaggccgctgcaaagtttggagcaggcgcagccggcgtgctcccaggagtaggaggtgcaggagtgcctggtgtgcctggagcaataccaggcattggaggaattgcaggagtgggtactcctgctgctgccgctgcggctgcagcagccgctaaagcagctaagtatggagccgccgcaggcctggttccaggaggcccaggctttggccccggagtagttggcgtccccggtgcaggagtcccaggagtgggagttcctggcgctgggattcctgtggttccaggtgcaggtattccaggcgctgcagtgcccggggtggtgagccctgaggctgcggctaaagccgctgccaaagctgccaaatatggagccagaccaggggtgggcgtcggaggtatccctacatatggtgtaggagcaggagggtttcccggttttggagtaggcgtgggagggattcccggcgtcgcaggagttcctggagtcgggggtgttcctggtgtgggaggagttccaggagtgggcattagtcctgaagcacaggctgcagccgcagcaaaggcagctaaatatggagtcggaacaccagctgcagccgcagctaaagccgctgcaaaggcagcacagtttggcttggtcccaggagtgggcgttgcacccggagtaggggttgcaccaggtgtgggagttgcccctggagtgggcctggcacccggagttggagtggccccaggtgtgggtgttgccccaggagttggcgttgcaccaggaattggacctggaggggtggccgccgccgccaaatctgctgccaaagttgcagcaaaagctcagcttagagcagccgctggccttggagcaggtatcccaggactaggtgttggagtgggcgttccaggactgggggttggagcaggagttcctggcttgggtgttggtgctggtgttcctggttttggcgctgttccaggagccttagctgctgcaaaggccgcaaaatacggcgcagccgtacctggcgtgcttggcggtctcggtgctctgggtggcgttggaattcctggcggagtcgttggagctggaccagctgctgcagctgctgctgccaaggctgcagctaaagcagcccagtttgggttagttggagccgctggattaggcggcttgggagttggaggattaggcgttcccggagtaggaggattaggcggcatcccaccagctgccgctgccaaggctgcaaagtatggagccgctggcttaggtggagtgttaggtggcgccggacaatttcctttgggaggagtggccgctagaccaggatttggattaagtccaatcttccctggaggagcctgtctgggaaaagcatgtggaaggaaaagaaaatga

SEQ ID NO: 5 - RNA, 2175 nt, synthetic construct
  source 1..2175: mol_type = other RNA
atggctggactgacagccgctgctcctagacctggtgttctgctgctgctcctgagcattctgcacccttctagaccaggcggagtgcctggtgctattcctggcggagttcccggcggagtgttttatcctggtgctggactgggagcccttggcggaggtgctcttggacctggtggaaagcctctgaaacctgtgcctggcggacttgctggtgcaggtcttggagccggacttggagcttttcccgccgtgacatttcctggcgctcttgtgccaggtggcgtggcagatgctgccgctgcttataaggctgccaaagccggcgctggactcggaggtgttcctggtgttggaggcctgggagtttctgctggtgctgtggttcctcaacctggcgctggtgttaagcctggcaaagttccaggcgttggactgcctggtgtttaccctggtggtgttctccctggcgctagattccctggcgttggagttcttcctggcgtgccaacaggtgccggcgtgaaacctaaagctcctggtgtcggcggagccttcgctggaatacctggcgtgggaccttttggcggacctcaaccaggtgtccctctgggctatcctatcaaggcccctaaactgccaggcggctacggcctgccttacacaactggcaagctgccctatggctatggacctggcggtgttgctggcgccgctggaaaagctggataccctactggaacaggcgtgggccctcaagcagcagctgccgcagcagctaaagccgccgctaaatttggagctggcgctgcaggcgttttgcccggcgttggcggagcaggcgtcccaggtgttccaggggcaatacctggaatcggaggaattgccggcgtcggaactccagctgcagcagccgcagccgccgctgccgcaaaagctgctaaatatggcgcagctgcaggcttggtcccaggcggacctggatttggaccaggtgttgttggagtgccaggcgctggcgtccccggcgtgggagttcctggtgccggaattcctgttgttcctggcgctggtattcctggcgctgctgttccaggtgttgtgtctcctgaagccgctgccaaggccgctgctaaggcagctaaatacggtgcccgaccaggcgtcggagttggcggaattccaacatatggtgtcggagccggcggattcccaggatttggagttggagtcggaggcatcccgggtgttgcaggcgttccaggcgtcggcggagttcctggcgttggtggtgttccaggcgtgggaatttctcctgaagctcaggccgctgccgctgccaaagcagccaaatatggcgtgggaacaccagccgctgctgctgctaaagccgctgcaaaagccgcacagtttggactggtgcctggtgtcggagttgctcctggcgtcggtgtcgcacctggtgttggtgttgcacccggtgttggattggctcctggcgtgggagttgcaccaggcgttggagtcgctccaggtgttggcgtggcacctggaataggtcctggtggcgttgccgcagctgccaaatctgcagcaaaggtggccgccaaagcacagctgagagctgctgccggtcttggcgctggaatcccaggactcggtgttggagtgggtgtccctggtcttggcgttggcgcaggcgtgccaggacttggagtcggtgctggcgtgcccggttttggagcagttcctggggcacttgctgcagccaaggctgctaagtacggggctgctgtgccgggtgtccttggaggattgggagcacttggaggcgttggtataccaggcggtgtcgttggagcaggacctgccgctgctgccgccgctgcaaaggctgcagctaaagctgctcagtttggcctcgtgggagccgctggacttggtggcctcggagtcggcggcttgggagtgcccggtgttggtggacttggaggaattccaccagccgccgcagcaaaagcagctaagtacggtgctgcaggactcggcggtgtcctcggcggagctggacaatttccacttggcggggttgccgccagaccaggattcggactgagccctatttttcctggcggcgcttgtctgggcaaagcctgcggcagaaagcggaagtaa

SEQ ID NO: 6 - DNA, 27 bp, synthetic construct
  source 1..27: mol_type = other DNA
ttggaccctcgtacagaagctaatacg

SEQ ID NO: 7 - DNA, 149 bp, synthetic construct
  source 1..149: mol_type = other DNA
ttttttttttttttttttttttttttttttttttttttttttttttttttttttttttttttttttttttttttttttttttttttttttttttttttttttttttttttttttttttttcttcctactcaggctttattcaaagacca

SEQ ID NO: 8 - RNA, 2175 nt, synthetic construct
  source 1..2175: mol_type = other RNA
atggcgggtctgacggcggcggccccgcggcccggagtcctcctgctcctgctgtccatcctccacccctctcggcctggaggggtccctggggccattcctggtggagttcctggaggagtcttttatccaggggctggtctcggagcccttggaggaggagcgctggggcctggaggcaaacctcttaagccagttcccggagggcttgcgggtgctggccttggggcagggctcggcgccttccccgcagttacctttccgggggctctggtgcctggtggagtggctgacgctgctgcagcctataaagctgctaaggctggcgctgggcttggtggtgtcccaggagttggtggcttaggagtgtctgcaggtgcggtggttcctcagcctggagccggagtgaagcctgggaaagtgccgggtgtggggctgccaggtgtatacccaggtggcgtgctcccaggagctcggttccccggtgtgggggtgctccctggagttcccactggagcaggagttaagcccaaggctccaggtgtaggtggagcttttgctggaatcccaggagttggaccctttgggggaccgcaacctggagtcccactggggtatcccatcaaggcccccaagctgcctggtggctatggactgccctacaccacagggaaactgccctatggctatgggcccggaggagtggctggtgcagcgggcaaggctggttacccaacagggacaggggttggcccccaggcagcagcagcagcggcagctaaagcagcagcaaagttcggtgctggagcagccggagtcctccctggtgttggaggggctggtgttcctggcgtgcctggggcaattcctggaattggaggcatcgcaggcgttgggactccagctgcagctgcagctgcagcagcagccgctaaggcagccaagtatggagctgctgcaggcttagtgcctggtgggccaggctttggcccgggagtagttggtgtcccaggagctggcgttccaggtgttggtgtcccaggagctgggattccagttgtcccaggtgctgggatcccaggtgctgcggttccaggggttgtgtcaccagaagcagctgctaaggcagctgcaaaggcagccaaatacggggccaggcccggagtcggagttggaggcattcctacttacggggttggagctgggggctttcccggctttggtgtcggagtcggaggtatccctggagtcgcaggtgtccctggtgtcggaggtgttcccggagtcggaggtgtcccgggagttggcatttcccccgaagctcaggcagcagctgccgccaaggctgccaagtacggagtggggaccccagcagctgcagctgctaaagcagccgccaaagccgcccagtttgggttagttcctggtgtcggcgtggctcctggagttggcgtggctcctggtgtcggtgtggctcctggagttggcttggctcctggagttggcgtggctcctggagttggtgtggctcctggcgttggcgtggctcccggcattggccctggtggagttgcagctgcagcaaaatccgctgccaaggtggctgccaaagcccagctccgagctgcagctgggcttggtgctggcatccctggacttggagttggtgtcggcgtccctggacttggagttggtgctggtgttcctggacttggagttggtgctggtgttcctggcttcggggcagtacctggagccctggctgccgctaaagcagccaaatatggagcagcagtgcctggggtccttggagggctcggggctctcggtggagtaggcatcccaggcggtgtggtgggagccggacccgccgccgccgctgccgcagccaaagctgctgccaaagccgcccagtttggcctagtgggagccgctgggctcggaggactcggagtcggagggcttggagttccaggtgttgggggccttggaggtatacctccagctgcagccgctaaagcagctaaatacggtgctgctggccttggaggtgtcctagggggtgccgggcagttcccacttggaggagtggcagcaagacctggcttcggattgtctcccattttcccaggtggggcctgcctggggaaagcttgtggccggaagagaaaatga

SEQ ID NO: 9 - RNA, 2913 nt, synthetic construct
  source 1..2913: mol_type = other RNA
atggcgggtctgacggcggcggccccgcggcccggagtcctcctgctcctgctgtccatcctccacccctctcggcctggaggggtccctggggccattcctggtggagttcctggaggagtcttttatccaggggctggtctcggagcccttggaggaggagcgctggggcctggaggcaaacctcttaagccagttcccggagggcttgcgggtgctggccttggggcagggctcggcgccttccccgcagttacctttccgggggctctggtgcctggtggagtggctgacgctgctgcagcctataaagctgctaaggctggcgctgggcttggtggtgtcccaggagttggtggcttaggagtgtctgcaggtgcggtggttcctcagcctggagccggagtgaagcctgggaaagtgccgggtgtggggctgccaggtgtatacccaggtggcgtgctcccaggagctcggttccccggtgtgggggtgctccctggagttcccactggagcaggagttaagcccaaggctccaggtgtaggtggagcttttgctggaatcccaggagttggaccctttgggggaccgcaacctggagtcccactggggtatcccatcaaggcccccaagctgcctggtggctatggactgccctacaccacagggaaactgccctatggctatgggcccggaggagtggctggtgcagcgggcaaggctggttacccaacagggacaggggttggcccccaggcagcagcagcagcggcagctaaagcagcagcaaagttcggtgctggagcagccggagtcctccctggtgttggaggggctggtgttcctggcgtgcctggggcaattcctggaattggaggcatcgcaggcgttgggactccagctgcagctgcagctgcagcagcagccgctaaggcagccaagtatggagctgctgcaggcttagtgcctggtgggccaggctttggcccgggagtagttggtgtcccaggagctggcgttccaggtgttggtgtcccaggagctgggattccagttgtcccaggtgctgggatcccaggtgctgcggttccaggggttgtgtcaccagaagcagctgctaaggcagctgcaaaggcagccaaatacggggccaggcccggagtcggagttggaggcattcctacttacggggttggagctgggggctttcccggctttggtgtcggagtcggaggtatccctggagtcgcaggtgtccctggtgtcggaggtgttcccggagtcggaggtgtcccgggagttggcatttcccccgaagctcaggcagcagctgccgccaaggctgccaagtacggagtggggaccccagcagctgcagctgctaaagcagccgccaaagccgcccagtttgggttagttcctggtgtcggcgtggctcctggagttggcgtggctcctggtgtcggtgtggctcctggagttggcttggctcctggagttggcgtggctcctggagttggtgtggctcctggcgttggcgtggctcccggcattggccctggtggagttgcagctgcagcaaaatccgctgccaaggtggctgccaaagcccagctccgagctgcagctgggcttggtgctggcatccctggacttggagttggtgtcggcgtccctggacttggagttggtgctggtgttcctggacttggagttggtgctggtgttcctggcttcggggcagtacctggagccctggctgccgctaaagcagccaaatatggagcagcagtgcctggggtccttggagggctcggggctctcggtggagtaggcatcccaggcggtgtggtgggagccggacccgccgccgccgctgccgcagccaaagctgctgccaaagccgcccagtttggcctagtgggagccgctgggctcggaggactcggagtcggagggcttggagttccaggtgttgggggccttggaggtatacctccagctgcagccgctaaagcagctaaatacggtgctgctggccttggaggtgtcctagggggtgccgggcagttcccacttggaggagtggcagcaagacctggcttcggattgtctcccattttcccaggtggggcctgcctggggaaagcttgtggccggaagagaaaaggtggaggcgggtccggcggaggcgggagcatggtgagcaagggcgaggaggataacatggccatcatcaaggagttcatgcgcttcaaggtgcacatggagggctccgtgaacggccacgagttcgagatcgagggcgagggcgagggccgcccctacgagggcacccagaccgccaagctgaaggtgaccaagggtggccccctgcccttcgcctgggacatcctgtcccctcagttcatgtacggctccaaggcctacgtgaagcaccccgccgacatccccgactacttgaagctgtccttccccgagggcttcaagtgggagcgcgtgatgaacttcgaggacggcggcgtggtgaccgtgacccaggactcctccctgcaggacggcgagttcatctacaaggtgaagctgcgcggcaccaacttcccctccgacggccccgtaatgcagaagaagaccatgggctgggaggcctcctccgagcggatgtaccccgaggacggcgccctgaagggcgagatcaagcagaggctgaagctgaaggacggcggccactacgacgctgaggtcaagaccacctacaaggccaagaagcccgtgcagctgcccggcgcctacaacgtcaacatcaagttggacatcacctcccacaacgaggactacaccatcgtggaacagtacgaacgcgccgagggccgccactccaccggcggcatggacgagctgtacaagtaa

SEQ ID NO: 10 - DNA, 21 bp, synthetic construct
  source 1..21: mol_type = other DNA
aagtggcattcaaggagtacc

SEQ ID NO: 11 - DNA, 21 bp, synthetic construct
  source 1..21: mol_type = other DNA
acgtggacaaaattggcttgc

SEQ ID NO: 12 - DNA, 23 bp, synthetic construct
  source 1..23: mol_type = other DNA
tacctgaaggccaaggagtacag

SEQ ID NO: 13 - DNA, 25 bp, synthetic construct
  source 1..25: mol_type = other DNA
cggaggtaacctgtaagtctgttaa

SEQ ID NO: 14 - DNA, 22 bp, synthetic construct
  source 1..22: mol_type = other DNA
cacacagacagccactcacctc

SEQ ID NO: 15 - DNA, 20 bp, synthetic construct
  source 1..20: mol_type = other DNA
ctgccagtgcctctttgctg

SEQ ID NO: 16 - DNA, 19 bp, synthetic construct
  source 1..19: mol_type = other DNA
gacttccaagctggccgtg

SEQ ID NO: 17 - DNA, 20 bp, synthetic construct
  source 1..20: mol_type = other DNA
ctccttggcaaaactgcacc

SEQ ID NO: 18 - DNA, 20 bp, synthetic construct
  source 1..20: mol_type = other DNA
tcaacagcgacacccactcc

SEQ ID NO: 19 - DNA, 20 bp, synthetic construct
  source 1..20: mol_type = other DNA
tgaggtccaccaccctgttg